European Patent Specification EP 3 132 028 B1, published October 25, 2023. Title: RECOMBINANT HOST CELL ENGINEERED TO OVEREXPRESS HELPER PROTEINS. Applicant: Boehringer Ingelheim Boehringer Ingelheim et al. The sequence listing filed with the application follows.

SEQUENCE LISTING (163 sequences)

SEQ ID NO: 1 - protein, 95 aa, Pichia pastoris
MLNKLFIAILIVITAVIGETTTSSTTASLSESPTLVWVTGTDASGRLATTQSAYTQQFSQLYSSIASPSSGSIGLGTIQGTVGIVRTYETITLAS

SEQ ID NO: 2 - protein, 86 aa, Pichia pastoris
MSTAIPGGQRTLAKRRAANLDKKQDEPTSARSAGAGGSSSTMLKLYTDEAQGLKVDPLIVLVLAVGFIFSVIGLHVVAKLTGKLIN

SEQ ID NO: 3 - protein, 361 aa, Pichia pastoris
MTPRSHIFFDISINNQPAGRIIFELFNDIVPKTAENFRALSTGEKGIGKSGKPLHYKGSTFHRIIKDFMVQGGDFTNGNGTGGESIYGEKFEDENFQLTHDKPFLLSMANAGPGTNGSQFFITTVPTPHLDNKHVVFGKVIAGKATVRKIERNSEGEAPIEPVVIEDCGELPEDADLTISDETGDKYEEVLKDNENIDIDDFEQVYQAITEIKELGTKYFKNGDTKIAFEKYQKAANYLLEYIPSDLSEEQSSKLELLKTSVFSNVALAGLKVSKFKDTIKYATLVIEDESADAKAKSKGYYRRGSAYSSLKDEDSAISDFQKALELSPGDPAISQSLQRTTKARKDRLAKEKAALSKFFE

SEQ ID NO: 4 - protein, 274 aa, Pichia pastoris
MSSDAVEQLENFQLIKFDRFDPSTQSTIRIARSPKPIPVKVVIVGDGGCGKTCLLNVFATGTFPEAYVPTIIENVVITLVTPTGQIAAVTLWDTAGQEEYDRLRPLSYSDVDVVLLCYSIDNLSTFHNVADKWYPEVAHFCPNTPIILVGTKSDMRRHQKSQPHFVSPQDSSQLARQMGAVMNIECSAKEVSNVNIVFDAAVSYCLSNSRPKTRGDNDNNRSNRRLSRAKRASMFIRGKDVSSTSGNSREELVEYDQDGLAIIPDRKKRKCSII

SEQ ID NO: 5 - protein, 127 aa, Pichia pastoris
MTNWKAILTPAQYQVLRLGGTERPYTGQYVNFKKNGTYLCSGCQTPLYKSGTKFDSSCGWPAFYEALPGAVKRIEDNSLGMRRIEIRCSKCDGHLGHVFEGEGFDTPTDSRHCVNSISLKFQGEEEN

SEQ ID NO: 6 - protein, 1027 aa, Pichia pastoris
MTTNGQKRQKTRKPLLINAFVMGCAGLQNPGLWKHPKDSSHRFNQIDHWTYLAKLAEKGKFNALFIADVLGGYDVYKGPENLATPAVAGAQWPVTEPSAVVSAMAAVTTNLAFGVTFSTISEAPYHFARRLSTLDHLTKGRIGWNVVSSYLESAARNLLNGEKLDEHDQRYLKAEEYIQIVYELLLSSWRDDAVVLDKKAGVYTDPTRFRKINFEGKFFKVPGPHIVDPTPQRLPVILQAGTSKVGKEFAAKHAEIVFVISFSPDDLKPKIAEVRQLAKEKFGRNHDDIKFVALATPVIGATHELAEEKYQELLSYGDIEGAQALFGGWTGIDLSQYGEDEELGNVSSNAMRGAVQNWTKAIPNEKRWTRKVIAKQITVGGLGPAFVGTPEEIADELEHWSDHAGLDGFNFTYAVNPLSFEEIVEDLIPVLQRRGLAQKEYPNPETGSTFRKNLFGTDFVPSTHPAYNLRWRAGVSKEEFEKSLNATTNWYSSFARSGALGELHNTCRILYLQIVKYKYRLRVRSEGNSIPFAKMTKENEAKRQKTSQPKAKKQLIINAFMSGSSGNQSPGLWSYPGDKSTEYTTLDYWVELAQKLEKAKFHSIFIADVLGGYDVYNGPGNYSAAAKSGAQFPMIEPSAAVTAMAAATKSITFGVTFSTISEAPYHFARRLGTLDLLTNGRVGWNIVSSYLDSAARNLLNGEPLPLHADRYKRAEEFLQVVYRLFLSSWRDDAYKLDKKTRTFADPKLIRTIDHVGEFFNVPGPQFLPPTPQRLPLILQAGTSKVGMDYAAKHAEVVFLASFDPESLQEKIKTVRDIAETKYNRPRDSIKFLILITVVIADTHEDAVKRYEDLASYADLEGAQALFSGWTGIDIGKYGEDEPLEHVESNAIKSHVKNWTKFKDNKPRARKDIAKQIGVGGSGPLLVGSVQEIADELERWAEVSDLDGFNFAYADYPQTFDDIIEKLLPELNKRGVFWDDYKIPGGTFRESVFGRKFVDKDHPAYDLRWRSDQTREEFEKKLAELEKK

SEQ ID NO: 7 - protein, 546 aa, Pichia pastoris
MSHLLLRDSFWGRTIYHLSKHRYFSFPEEKDGFIAPEKYYLNMDQVSIHAESEKNIVEGLVDTSNSSLEEVKTTRVIVDWDEYDQKENPQNWSSLLKCFVVFEVGILTVAVYMGSAIYTPGIEDIMRDLNVSRTVATLPLTLFVIGYAVGPMIFSPMSEHPAIGRTTIYVWTLFIFAILQIPTALTTNIAGFCILRFIGGFFASPALATGPASVGDVIAIPHLPVGLGLWSICAVCGPSLGPLFGAIFSQLVSWRWCFWFLLITSGTLFIVLGFTLPETYVPTLLYRKARRLRALTKNELIISKGELDIQDRTAKEVLIECLWRPVDISFRDPVVLMINLYISMVYSIWYIWFEAFPIVFLEIYGFSLIGMGASFAGILIGVLICSACYCYACHVTFARRIIANETIHPEFFVPGAIIGGCIMPTGIFILGWTATKSVHWIVPIIGSGLFAAGGYLIFQTLFNYLAMSFPRYMASAFAGNDLFRSFSASVFPLFGHALYANLGSEKFPVGWGSSVLGFITVAMIAIPVTFMRYGPRLRANSRYAGP

SEQ ID NO: 8 - protein, 355 aa, Pichia pastoris
MTDYVTSKRPDNVLNWTSIHVSSWIGETIPEIDPSLLQNFLEHDIAGDVLPYLKSEDLKEIGINELKHRISIKKNIHELLVSNEKHIDTSILSDTATELGTLILTNKFITQMANRKNVVDDSTHHSNNRRLTEQFNKLRKDLLPIFKWIKETQPLPTPENTHFANMGSVPASPVEHTSGESTLSNPSLSTINAGEGVNSAVAGQSLGRKPTLSSRRQSHALSPTGEHLNVSSSSPSTGNFETLNGERPNLRSASSGSQEHTENELLKPLRVKADEPCYKVIQNAMKRHGLSVDDWRKYALVICYGDEERVLGLHEKPGSIFKELKDQKQNPAIMLRQIDTNNDDQNHIETPGGRL

SEQ ID NO: 9 - protein, 194 aa, Pichia pastoris
MRFSNVVLTAIAAAGVQADEALYTVFYNDVTENAQEYLSYIQANTAAGFTDLLSLYTELATYTDDSYTSIFTEEDFPASELSSFVVNLPWYSSRIEPQVAAAETGESEEESETGESEEESETGEETETETGSESESESESETSATGTGTGTSASESAETETSTDAAVSIDHPKSTLLMGLTAAVVSITFGVFAL

SEQ ID NO: 10 - protein, 806 aa, Pichia pastoris
MNKPNGSEQQPPSRGMKQESGGPVTSSTTPGTNTGLENSHSMGADMEPDVGATSPRHLLNGYIYDYLVKSNMQNLADQFAQETELLETDLTVPMDTPSGYLLEWWMVFWDLFNARLKQRGSQKAHQYIQLNMLRQQQQRTMRNTARVQKVPLRPHTQSSPSMSQTFIPQQPQQQAQGQQHAQAQAQVQAHQQAQHHAQAQVPVQPQQHQLGGQTQQQQSINTGSPAGPNAINSRVQHLAQQQMNHLRQQATATTQQPIPQQNIPSNQQGPTGPYPTSPSRRPRLLSNESGASAPSVMTKSQLQGVPPSQQPHQQQGQQVGPPNQHQGQSSSFYSGMPPQGVVVPHQFNPQQYANMLARQQHVQAQQQVQLQQVQHVQQRQQQDQQQHRLSAGSPGHPSFGVFQQPPPMSNHNQVMINQQGETFFDPHSPYAQPNGYPQPQQQQQQQQQQQQQQQPQQQQQQQQQQKQQPPPPPRQPQRQQAMAMAPLPHSTSAAGTPHSSTTPRFSQPGPVYQQPLPASQPQHSPPSSIQQPELVPTPGSQHQQIAQPQSQSQHQQSQQSQSSASKIVGIQEYQKELMMLEKQNKQRHDMACKKGSGHFSNFDPIPEHTPPEPKFNVNVMLPPQNSAVVTKNTPGTSPGTQTQNTAHSTGNTSAGSTPNNVAPVRKKKEPAKKKAKKATEPPTPTTPQTPIAARTHQNSTGGIPGNNAATKRRKREPLVDQTVSPNLNEASKSTKTGKISSQTDFTGSDNGFLQDFGDGTGPPTGTDDMEFDFNSFLNNETGEPNSSTIHFDNVFNWGEGTEAGDL

SEQ ID NO: 11 - protein, 149 aa, Pichia pastoris
MVVHNPNNWHWVDKNCLPWAKSYFQEVLPNTTQKNDAYEIVVTSVDLVDGDCDVTQRKGVTKCIFDLKIQVSATVKVNTNSEVEEISYTVTLPELVHDQDEDEYEYVIEGNLDHKSQIRKLLTPLLTEKLSKFQQALIDAHTQDVQHST

SEQ ID NO: 12 - protein, 354 aa, Pichia pastoris
MKIWLVLLLVFATVFAETDYYKVLGVAKNADEKDIKKAYRSLSKKFHPDKNPGDDEAAQKFIQVGEAYDVLGDPEKRQRYDRFGAEGLDSRQEQFHDPFDMFQQFFGGGGQQHRGKPKGKSSLLHLEFSLQDFYNGASNDFRIEMQNICETCSGSGSQDGKVHQCDTCKGHGRVVQTRQFGGGMQQRFETICPKCSGTGNLITHKCKKCQGNRVVRGPRIHNVHLGAGTSRNHVEILEGQGDQSPDWIAGDLQIMFKEKAEGNMGYRRIGNNLYRDEALTLKEALHGGWERQIAFLDKIENTITLSKKKGEVVVDGQVDTIKGRGMPLHDHYDEHGDLFIKYHIIYPQQIRDEL

SEQ ID NO: 13 - DNA, 288 bp, Pichia pastoris
atgttaaacaagctgttcattgcaatactcatagtcatcactgctgtcataggcgagacgactacgtcatctaccactgccagtctctccgaaagccctactctggtttgggtgactggcactgatgcaagtgggagattggcaactacacagtctgcttacactcaacagttttcacagttatactcatccatagcatctccatcaagtggtagcataggcctgggtactatccaggggactgttggaattgtcagaacatatgagacaattacccttgccagctaa

SEQ ID NO: 14 - DNA, 261 bp, Pichia pastoris
atgtctacagcaattccaggaggacagagaacgttagctaaaagaagagcagcaaacttggataagaaacaggatgaaccaacctccgccagatctgccggtgctggaggttcttcgtctaccatgctaaagttgtacacagacgaggcccaaggtttgaaagttgatcctttaattgttcttgttcttgctgttggtttcattttcagtgtcattggtttgcacgttgttgctaagctgacaggaaagttgatcaactaa

SEQ ID NO: 15 - DNA, 1086 bp, Pichia pastoris
atgactccccgttctcatattttctttgacatctccatcaacaaccagccagctggcagaataatctttgagctcttcaatgacattgttcctaagacagcagagaattttagagctttatctactggtgagaaaggtataggtaagtctgggaaaccattgcactacaagggttctactttccataggatcattaaggattttatggtacaaggtggtgactttaccaacggtaacggtactggaggcgaatccatatatggagaaaaatttgaagatgaaaatttccaattgactcatgacaaaccgttccttctctctatggcaaacgctggaccaggaactaatggatcccagttttttatcaccaccgttcctactcctcatctggataacaagcatgtagtgtttggaaaagtaattgctggtaaagccacagttagaaagattgaaagaaactccgaaggtgaagctccaattgaacccgttgtcattgaggactgtggtgaacttccagaagacgcagatttgaccatctccgacgagactggagacaagtatgaggaagttctgaaagataatgagaacatagacatcgatgactttgaacaggtctaccaggccatcactgaaatcaaagaattgggtacaaagtatttcaaaaatggtgacaccaaaatcgccttcgaaaagtatcaaaaggctgctaattatttgctggaatacataccatcagatttatcagaggaacagagctctaagttggagctgctaaaaacatctgtcttctccaacgtggcattggctggactgaaagtttccaagttcaaagacacgattaagtatgccacattggtcattgaggatgaatctgcggatgcaaaggccaagtccaaaggctactaccgtagaggaagtgcttacagctcactgaaagacgaagattcagccatctcagatttccagaaagcacttgaattatccccaggtgatcctgcaattagccaatctctacaaagaaccacgaaggccagaaaagaccgtcttgccaaagagaaagctgctttgtctaagttctttgagtag

SEQ ID NO: 16 - DNA, 825 bp, Pichia pastoris
atgtcgtctgatgctgtggagcaacttgaaaacttccagttgatcaagttcgacagattcgatccttcaacgcaatcgactatcagaatagcgcgatctcccaaaccaattccagtcaaggttgtgatagtgggagatggtggatgtggaaagacatgtcttctcaatgtctttgccactggaacgtttcctgaggcgtatgtccccacaatcatagaaaatgtggttattacattggtgaccccaactggccagatagctgccgttactctgtgggatactgcagggcaagaagagtacgacagattgagacccctaagctactccgacgttgacgtggtcttgctgtgctacagcatagacaatctgtccacctttcataatgtggccgacaaatggtacccagaagtggcacatttttgtccaaacacaccgatcatcttggtaggtaccaaatctgatatgcggcgtcatcagaagagtcagccgcactttgtatctccccaggattcgtcgcagttggcaaggcagatgggggcagtgatgaacatcgagtgttctgcgaaggaggtttcaaacgtcaatatcgtttttgatgctgctgtgtcgtactgtttgagtaacagcaggcccaagaccagaggggataatgacaacaataggagtaacagacggctaagtagagccaagcgagccagcatgtttataaggggtaaggatgttagctcaacgtcaggaaactctcgggaagaacttgttgaatacgatcaagatgggttggcaataataccggacagaaagaaacgcaaatgtagcattatttga

SEQ ID NO: 17 - DNA, 384 bp, Pichia pastoris
atgactaactggaaagcgatattgactcccgctcaataccaagtcctccgtttgggcggaacagaaagaccgtataccggacagtatgtgaacttcaagaaaaatggaacctacttgtgtagtgggtgtcaaactccgctttacaaaagtggcacaaaatttgattcatcttgtggttggcctgcattctatgaagcattacctggagcagttaaacgaatagaagacaattcgcttggaatgcgaagaatagaaatcagatgctccaaatgtgatggacatcttggccatgtttttgagggtgagggatttgacactccaacagattccagacattgtgtcaacagcatcagcctaaaatttcaaggtgaagaagagaactaa

SEQ ID NO: 18 - DNA, 3084 bp, Pichia pastoris
atgactacaaacggccagaaaagacaaaaaactcgcaaaccacttttgatcaacgcatttgtcatgggatgtgctgggttacagaatcctggtttatggaagcatcccaaggactcatcccatagatttaatcagattgatcactggacttatttggccaagttagccgaaaaggggaagtttaatgcgctcttcattgccgacgtcttgggtggctatgatgtctacaaaggacctgagaatttagccactcctgctgtggctggagcccagtggcctgtcaccgagcccagtgctgtggtctccgccatggctgcagtcacaactaacttggcgtttggagtgacgttctctactatcagcgaagccccctatcattttgccagaagactgtccactttagaccacttgaccaagggtagaataggatggaatgttgtttcatcttacttggagagtgctgctcgtaacctcttgaatggtgaaaaattggacgagcatgaccaaagatacttgaaagctgaagagtacattcaaatagtttatgagctgttgttatcgtcttggagagatgatgcagtagttttagacaagaaagctggtgtttatactgacccaacaagatttcgaaagatcaactttgaaggtaaatttttcaaagttccgggaccacatattgttgaccccacccctcaaagactgcctgtgattcttcaagctggtacttctaaagttggtaaggagtttgctgctaagcatgccgagattgtgtttgtcatttcattttctccagatgatttgaaacccaagattgcagaagttcgtcaactggccaaagaaaagtttggtagaaaccacgacgatattaagtttgttgcccttgcaacccctgttattggagccacacatgaactagctgaagaaaagtaccaagagttactaagttatggtgatattgaaggtgctcaagccttatttggagggtggactggcattgacctctctcaatatggcgaagatgaagaactaggaaatgttagttccaatgctatgcgtggcgctgtacaaaactggactaaagcaattccaaatgagaagcgttggacacgtaaggttattgctaaacagattaccgttggtggtctaggtccagctttcgttggaaccccagaagaaatcgccgatgagctggaacactggtccgaccacgctggtttggacggattcaacttcacttatgctgtcaacccgctttctttcgaagagatagtggaagacttgattccagttcttcagcgaagagggttggcccaaaaggaatacccaaatccagaaactggaagcacattccgtaaaaacctttttggaacagactttgtaccatctacccacccagcttataacttaagatggagggctggtgtgtccaaggaagaattcgaaaagtccctaaacgccacaacaaattggtattccagtttcgctaggtcaggtgctctaggtgaattgcataatacatgcaggattctctatctccaaatagtgaaatataaatataggcttcgagtccgttcagaagggaatagcatccccttcgccaaaatgaccaaggaaaatgaagccaagaggcagaaaacctctcaaccaaaagcgaagaagcaattgattatcaatgctttcatgtcaggctcttcgggtaaccaatcgccaggactgtggtcgtaccctggagacaaatcaacagagtatactaccctagattactgggtggagttagctcaaaagctggaaaaggccaaattccattctatcttcattgccgatgttctgggtggatatgacgtttacaatggacctggaaactacagtgctgctgcaaaatctggtgcccaatttccaatgattgaaccaagtgctgcagttactgccatggctgctgctaccaagtcaataacgttcggagtgactttttccactataagtgaggcaccttatcattttgcaagaagattgggaactttagatctgctgacaaacggaagagtcggctggaatatcgtctcttcgtatcttgacagtgccgccagaaatcttttgaatggagaaccactccctctccatgcagaccgttataagagagccgaagaattcctacaagttgtatatcggttattcctttcttcatggagagacgatgcttataaattggataagaaaaccagaacctttgctgacccaaaacttattagaactatcgaccacgttggagagttcttcaatgtcccaggcccccagttcctaccacccactcctcagagactaccgctgattttgcaggctggtacttccaaggttggtatggattatgctgcaaaacatgcagaggttgtctttttagcttcatttgacccagagtcactccaagaaaaaatcaaaacagtgagagatatcgctgaaaccaagtacaacagaccaagagattcaatcaaattcttaattttgataacagtagtcatagctgatacacacgaagatgccgtgaagagatacgaagatctcgccagttatgctgatctggaaggggcccaagcactgttcagtggttggactggaatagatattggaaagtatggtgaagatgaacctcttgagcatgtggaatctaacgctattaagagccatgttaagaactggactaagttcaaggacaataagcctagagccagaaaagatatcgctaaacagattggagttggaggctcaggtcccttacttgttggatctgtacaagagatagccgacgagcttgagagatgggcagaagtctctgacctcgatggctttaacttcgcttacgcagattacccccaaacttttgatgatatcattgaaaaactgcttccagagttgaacaagagaggtgtgttctgggatgattataaaattccaggtggaaccttcagagagagcgtgtttggaagaaagttcgttgataaggatcatcctgcttatgatctgagatggagaagtgaccaaactagggaggagtttgaaaagaaactggctgaattggagaaaaaataa

SEQ ID NO: 19 - DNA, 1641 bp, Pichia pastoris
atgtctcatctattactgcgtgacagcttttggggaaggaccatctaccatctgagtaaacacaggtatttctcttttcctgaagagaaagatggtttcattgctcctgaaaagtactacctgaatatggaccaagtatcgatacatgctgaatctgagaaaaatatagtggaaggtttggtagacacttcaaattcttcgttggaggaagtaaagaccactagagtcatagtcgactgggatgaatatgatcagaaagaaaatccccaaaactggagctcgcttttaaagtgcttcgttgtttttgaagtgggaatcttaaccgtagctgtttatatgggatctgcaatttacactcccggtatagaagatattatgagagatctcaatgttagcagaacggtggcaacacttccattaaccttgtttgtgattggatacgctgtgggtccaatgatattctcccccatgtctgagcatcccgctatcggaaggacaacgatatatgtgtggaccctgttcatatttgctatactacaaatcccaacggccctgaccactaacattgctggattttgcattttgaggtttattggagggttttttgcgtcaccagcattagctacaggtccagcttctgtaggtgatgttattgcaatcccgcacttgcctgtagggttaggcctttggagtatctgtgctgtttgtggtccttctctaggaccactttttggagccatattttcccaacttgtgagttggaggtggtgcttctggtttctgttaattacctctgggacactatttatagttcttggcttcactttaccagaaacgtatgtaccaacccttctttacagaaaggctaggaggctacgagcattaacaaaaaacgaactgattatcagcaaaggggagttagatattcaggacagaactgccaaggaagttttgattgaatgcttatggaggccagtcgacatatcattcagagaccccgttgtcttgatgataaatctttacatttcaatggtttattctatttggtacatttggtttgaagcgtttcctattgtattcttagagatatatggattcagccttattggaatgggagctagttttgccggaatcttaattggtgtcttaatatgctctgcgtgctattgctatgcgtgtcatgttacttttgcaagaagaataattgcaaacgaaaccattcatcctgagttctttgtaccgggcgctattattggaggttgcataatgcccactggaatctttattttgggatggactgccaccaaaagtgtccactggattgtacctataataggtagcggtttatttgctgctggtggttatctcattttccagacactcttcaactaccttgcaatgtctttccctagatacatggcatcagcttttgccggaaatgatcttttcaggtccttttctgccagtgttttcccactgtttggacatgcactatatgccaacttgggatccgaaaagttccctgttggttggggttcttctgtactggggttcatcactgttgcaatgatcgcaattccagtaactttcatgagatatggtccaagattgcgtgcaaattctagatatgccgggccatga

SEQ ID NO: 20 - DNA, 1068 bp, Pichia pastoris
atgacggactatgtcacttctaagcggccagataacgtgctcaattggacaagtattcatgtatcgtcctggataggggagactattcctgagatcgatccaagtctactccaaaattttttagaacatgacattgcgggagatgttctaccctacttgaagtctgaagatctgaaggaaattgggatcaacgagctcaagcacagaatctctataaaaaagaacattcatgaacttcttgtgagcaatgaaaagcacattgataccagtattctatcagacaccgctaccgagctaggaactttgatactgactaataaattcataacccagatggcgaacagaaagaatgttgtagatgattccactcatcattcgaataacagaaggctcactgaacagtttaataagcttcgcaaagatcttttgccgatattcaaatggatcaaggagacccaaccattacccactccagagaatacacatttcgcaaatatgggttcagtaccagcatctcctgtggagcatacttcaggtgagtcaacattgtctaaccccagtctaagcaccatcaatgctggcgaaggagtgaactctgcagttgcagggcaatctctcgggaggaaacctacattatcctccagaagacaatcacatgctttgtctccaactggtgaacacctgaatgtgtcatcatcatctccttcgacggggaattttgaaactctgaatggagaaagacccaatcttagatctgcttcgtcaggatcacaggaacatactgagaacgaactattgaagccgttgagagttaaagcagatgagccttgctataaggtgattcagaatgccatgaaaagacatggcttatcggtagatgattggcgcaagtatgctttggtcatctgctatggagatgaagaacgagtactaggcttacatgaaaaacctgggagtatcttcaaggaactcaaagatcagaaacagaatcctgcaatcatgcttcgtcaaattgacactaataatgacgatcagaaccatattgaaacccctggagggagattatga

SEQ ID NO: 21 - DNA, 585 bp, Pichia pastoris
atgagattttctaacgtcgttttaactgcaattgccgctgccggcgtacaggcagatgaagccctttacactgtgttctacaatgatgtcactgagaacgcccaagagtatctgtcttacatccaggccaatactgcggctggtttcactgacctcttgagtctgtacactgaactggccacttacaccgacgattcttacacaagtatctttactgaggaggatttccctgcgagcgaactttcatcgttcgttgttaacctgccatggtattcctccagaattgagccacaagttgcggctgctgaaactggtgaaagtgaggaggaatcagagactggtgaaagtgaggaagaatcagagactggtgaggagacagaaactgagactggatctgagtctgaatctgagtctgaatcggagacctccgctactggcactggcactggcacctccgcctctgagagcgcggagactgaaacttctaccgacgctgctgtgtctatcgatcacccaaagtccaccttattgatgggtttgactgccgcagttgtcagtatcactttcggagtctttgccttgtaa

SEQ ID NO: 22 - DNA, 2421 bp, Pichia pastoris
atgaacaagccaaacgggtctgaacaacaaccaccgtcacgcggaatgaagcaagagtcaggaggcccagttacttcatctacgacgccgggtaccaatactggcctagaaaactctcattccatgggggcggatatggagcctgatgttggtgctacctctcctcgccatcttcttaatgggtacatttacgattatttagtcaaatctaacatgcaaaatttggctgatcaatttgcccaagagacggagctcttagaaacagacttgacagtaccaatggatacgccttcaggctatcttctagaatggtggatggtattctgggaccttttcaatgcccgcctaaagcaacggggttcacagaaggcccaccagtatattcagttgaacatgctacgacaacagcaacagaggaccatgcgaaatacagcccgtgttcaaaaagtcccgttgaggccacacacccaatcatctccttcaatgtcacagacttttattccacagcagcctcaacagcaagcacagggacaacagcacgcccaggctcaagcccaagtgcaagcacatcagcaagcccaacaccacgcgcaggcacaagtgccagtgcaaccgcaacagcaccagctaggaggccaaactcaacagcagcaatccattaacactgggtctcctgcgggtccaaatgctatcaactcgcgtgttcaacacttagcacaacaacagatgaatcaccttcgccagcaggcgactgccactacgcaacaacctatcccgcaacagaatatcccatcaaaccaacagggtcctacaggcccttatcctacttccccttcaagaagaccgagattactgtctaacgaatcgggtgcaagtgcaccctctgtaatgacaaagtcacagctccaaggagtccctccctcacaacaaccacaccagcagcaaggtcagcaggtaggcccccctaatcaacatcaaggtcaatcttcttccttttattcgggcatgcctcctcaaggggtcgtggttcctcatcagttcaatcctcagcagtatgccaatatgctagcaagacaacagcatgtacaagctcaacaacaggttcagttacaacaggtccaacatgtacaacagagacaacagcaagaccaacaacaacaccgcctgtccgccggttcaccggggcacccttcatttggcgtttttcaacaacctcctccgatgtcaaaccataatcaggtcatgatcaatcagcagggagaaactttttttgatccacattctccatatgctcaacctaacgggtacccccagccacagcaacaacaacaacaacagcaacaacaacaacaacagcagcaaccgcaacagcagcagcagcagcagcagcaacagaagcagcaaccaccaccaccaccacgacagcctcagcgccaacaagcgatggccatggctcctctgcctcactctacttctgccgccggtactcctcactcgtccaccacacctagattctcgcaacctggtcctgtttatcagcagcctttacctgcatctcaaccgcaacattctccgccttcttctattcagcagccggagctagttccaactccagggtcacaacatcagcaaatagcacaaccacaatcacagagccaacaccagcaatcgcaacagtctcaatcaagtgcttctaaaattgtaggtatacaggagtatcagaaagagctaatgatgcttgagaaacagaacaaacagcgtcatgacatggcatgtaagaagggaagcgggcatttttctaactttgatccaattccagagcacacaccgcccgaaccaaaatttaatgtgaatgtaatgctccctccccagaactctgcagtggtcacgaagaatactcccggaacttcacctggtacacaaactcaaaacactgcacatagtactggtaacacttctgcggggtctacaccaaataatgtcgcacctgtacgaaagaaaaaggagccagctaaaaagaaggcaaagaaagctactgagcccccgactcccactactccacagactccaattgcagctaggacacatcaaaactctacaggcggcattcctggtaataatgctgctactaagcgacgaaaacgggagccgctggttgatcaaactgtttcacctaaccttaacgaagcttccaagtcaacaaagaccggaaaaatttcatctcaaactgactttacaggttctgacaatggattcttacaggattttggcgatggaactggtcctcccactggaaccgatgatatggaatttgattttaacagttttcttaataacgaaactggcgaacctaatagttcaaccattcattttgacaatgtattcaattggggagaaggtaccgaagccggagatttatag

SEQ ID NO: 23 - DNA, 450 bp, Pichia pastoris
atggtggtgcacaaccctaataactggcactgggtcgacaagaactgccttccttgggccaaaagctactttcaggaagtccttccaaacaccactcagaagaatgacgcctatgaaatagtggtaacatctgtggaccttgtagatggagactgcgatgtcactcaacgtaaaggtgttaccaaatgtatttttgatctgaagatacaggtatctgcaaccgtcaaagtcaacacgaacagtgaagtagaggagatcagttatacagtgacattacctgaactggtgcacgaccaggacgaggatgaatatgaatacgtaatagagggaaatttggatcacaagtctcaaattagaaagctactcactcctctgttgaccgagaagttatcaaagtttcaacaagctttgatagacgctcatactcaggatgttcagcatagtacctag

SEQ ID NO: 24 - DNA, 1065 bp, Pichia pastoris
atgaagatatggctggtacttcttttagtttttgccacggtgtttgccgagacagattattataaagttcttggagtagctaaaaatgcggatgaaaaagatatcaagaaggcctacagatcgttgagtaagaagtttcatccagataagaacccgggtgatgatgaagccgctcaaaagttcattcaagttggagaagcttatgatgtgcttggtgatcccgagaagcgtcaaaggtatgacagatttggagcagaaggactggactcaagacaggaacaattccatgatccatttgacatgtttcaacagttcttcggaggaggtggacagcaacacagaggcaaaccaaagggtaagagttccttgttacatttagaattcagtctacaagacttttacaatggtgctagtaacgactttagaatcgaaatgcagaatatctgtgaaacttgttctggatcaggttcacaagacgggaaagttcatcaatgtgacacttgcaaagggcacgggcgtgttgttcaaacgagacagtttggtggtggcatgcaacagaggtttgaaacaatttgcccaaaatgttcaggaacaggaaatctgatcactcacaagtgtaagaaatgccaaggaaaccgtgtagttagaggacccagaattcacaatgtgcatttgggggcgggaactagtaggaaccatgttgagatcctggaaggtcagggagaccagtctccagactggattgcaggtgatctacaaatcatgttcaaggagaaagccgaaggcaacatggggtatagaagaataggaaacaacctgtacagagacgaagcattaacgctgaaagaggcattgcatggtggctgggagagacaaattgcgtttttggataaaatagagaacacgattactctttccaagaagaaaggagaggtggtagttgacggccaagtagacaccatcaagggtagagggatgccattacatgaccactatgacgaacatggtgatctctttatcaagtaccatatcatttacccgcaacaaattagagacgaattgtga

SEQ ID NO: 25 - protein, 312 aa, artificial
  Synthetic Construct
MRFPSIFTAVLFAASSALAAPVNTTTEDETAQIPAEAVIGYSDLEGDFDVAVLPFSNSTNNGLLFINTTIASIAAKEEGVSLEKREVQLVQSGGGLVQPGGSLRLSCAASGFTFSHYWMSWVRQAPGKGLEWVANIEQDGSEKYYVDSVKGRFTISRDNAKNSLYLQMNSLRAEDTAVYFCARDLEGLHGDGYFDLWGRGTLVTVSSASTKGPSVFPLAPCSRSTSESTAALGCLVKDYFPEPVTVSWNSGALTSGVHTFPAVLQSSGLYSLSSVVTVPSSSLGTKTYTCNVDHKPSNTKVDKRVESKYGPP

SEQ ID NO: 26 - protein, 299 aa, artificial
  Synthetic Construct
MRFPSIFTAVLFAASSALAAPVNTTTEDETAQIPAEAVIGYSDLEGDFDVAVLPFSNSTNNGLLFINTTIASIAAKEEGVSLEKRAIQLTQSPSSLSASVGDRVILTCRASQGVSSALAWYQQKPGKAPKLLIYDASSLESGVPSRFSGSGSGPDFTLTISSLQPEDFATYFCQQFNSYPLTFGGGTKLEIKRTVAAPSVFIFPPSDEQLKSGTASVVCLLNNFYPREAKVQWKVDNALQSGNSQESVTEQDSKDSTYSLSSTLTLSKADYEKHKVYACEVTHQGLSSPVTKSFNRGEC

SEQ ID NO: 27 - DNA, 939 bp, artificial
  Synthetic Construct
atgagattcccatctattttcaccgctgtcttgttcgctgcctcctctgcattggctgcccctgttaacactaccactgaagacgagactgctcaaattccagctgaagcagttatcggttactctgaccttgagggtgatttcgacgtcgctgttttgcctttctctaactccactaacaacggtttgttgttcattaacaccactatcgcttccattgctgctaaggaagagggtgtctctctcgagaagagagaggtccaattggtccaatctggtggaggattggttcaaccaggtggatctctgagattgtcttgtgctgcttctggtttcaccttctctcactactggatgtcatgggttagacaagctcctggtaagggtttggaatgggttgctaacatcgagcaagatggatcagagaagtactacgttgactctgttaagggaagattcactatttcccgtgataacgccaagaactccttgtacctgcaaatgaactcccttagagctgaggatactgctgtctacttctgtgctagagacttggaaggtttgcatggtgatggttacttcgacttatggggtagaggtactcttgtcaccgtttcatctgcctctaccaaaggaccttctgtgttcccattagctccatgttccagatccacctccgaatctactgcagctttgggttgtttggtgaaggactactttcctgaaccagtgactgtctcttggaactctggtgctttgacttctggtgttcacacctttcctgcagttttgcagtcatctggtctgtactctctgtcctcagttgtcactgttccttcctcatctcttggtaccaagacctacacttgcaacgttgaccataagccatccaataccaaggttgacaagagagttgagtccaagtatggtccaccttaa

SEQ ID NO: 28 - DNA, 900 bp, artificial
  Synthetic Construct
atgagattcccatctattttcaccgctgtcttgttcgctgcctcctctgcattggctgcccctgttaacactaccactgaagacgagactgctcaaattccagctgaagcagttatcggttactctgaccttgagggtgatttcgacgtcgctgttttgcctttctctaactccactaacaacggtttgttgttcattaacaccactatcgcttccattgctgctaaggaagagggtgtctctctcgagaagagagctatccagttgactcaatcaccatcctctttgtctgcttctgttggtgatagagtcatcctgacttgtcgtgcatctcaaggtgtttcctcagctttagcttggtaccaacaaaagccaggtaaagctccaaagttgctgatctacgacgcttcatcccttgaatctggtgttccttcacgtttctctggatctggatcaggtcctgatttcactctgactatctcatcccttcaaccagaagactttgctacctacttctgtcaacagttcaactcttaccctttgacctttggaggtggaactaagttggagatcaagagaactgttgctgcaccatcagtgttcatctttcctccatctgatgagcaactgaagtctggtactgcatctgttgtctgcttactgaacaacttctacccaagagaagctaaggtccaatggaaggttgacaatgccttgcaatctggtaactctcaagagtctgttactgagcaagactctaaggactctacttactccctttcttccaccttgactttgtctaaggctgattacgagaagcacaaggtttacgcttgtgaggttactcaccaaggtttgtcttctcctgttaccaagtctttcaacagaggtgaatgctaa

SEQ ID NO: 29 - protein, 303 aa, artificial
  Synthetic Construct
MRFPSIFTAVLFAASSALAAPVNTTTEDETAQIPAEAVIGYSDLEGDFDVAVLPFSNSTNNGLLFINTTIASIAAKEEGVSLEKRDVQLQESGPSLVKPSQTLSLTCSVTGDSITSDYWSWIRKFPGNRLEYMGYVSYSGSTYYNPSLKSRISITRDTSKNQYYLDLNSVTTEDTATYYCANWDGDYWGQGTLVTVSSASTKGPSVFPLAPSSKSTSGGTAALGCLVKDYFPEPVTVSWNSGALTSGVHTFPAVLQSSGLYSLSSVVTVPSSSLGTQTYICNVNHKPSNTKVDKRVEPKSCDK

SEQ ID NO: 30 - protein, 299 aa, artificial
  Synthetic Construct
MRFPSIFTAVLFAASSALAAPVNTTTEDETAQIPAEAVIGYSDLEGDFDVAVLPFSNSTNNGLLFINTTIASIAAKEEGVSLEKRDIVLTQSPATLSVTPGNSVSLSCRASQSIGNNLHWYQQKSHESPRLLIKYASQSISGIPSRFSGSGSGTDFTLSINSVETEDFGMYFCQQSNSWPYTFGGGTKLEIKRTVAAPSVFIFPPSDEQLKSGTASVVCLLNNFYPREAKVQWKVDNALQSGNSQESVTEQDSKDSTYSLSSTLTLSKADYEKHKVYACEVTHQGLSSPVTKSFNRGEC

SEQ ID NO: 31 - DNA, 915 bp, artificial
  Synthetic Construct
atgagattcccatctattttcaccgctgtcttgttcgctgcctcctctgcattggctgcccctgttaacactaccactgaagacgagactgctcaaattccagctgaagcagttatcggttactctgaccttgagggtgatttcgacgtcgctgttttgcctttctctaactccactaacaacggtttgttgttcattaacaccactatcgcttccattgctgctaaggaagagggtgtctctctcgagaagagagacgttcaattgcaagaatctggtccatccttggttaagccatcccagactttgtccttgacttgttccgttactggtgactccatcacttctgactactggtcctggatcagaaagttcccaggtaacagattggagtacatgggttacgtttcttactccggttccacttactacaacccatccttgaagtccagaatctccatcactagagacacttccaagaaccagtactacttggacttgaactccgttactactgaggacactgctacttactactgtgctaactgggacggtgactattggggtcaaggtactttggttactgtttcctccgcttccactaagggtccatctgtttttccattggctccatcctccaagtctacttcaggtggtactgctgctttgggttgtttggttaaggactacttcccagagccagttactgtttcttggaactccggtgctttgacttccggtgttcacactttcccagctgtcttgcaatcctccggtctgtactccttgtcctccgttgttactgttccttcttcctccttgggtactcaaacttacatctgtaacgttaaccacaagccatccaacactaaggttgacaagagagttgagccaaagtcctgtgacaagtaatag

SEQ ID NO: 32 - DNA, 903 bp, artificial
  Synthetic Construct
atgagattcccatctattttcaccgctgtcttgttcgctgcctcctctgcattggctgcccctgttaacactaccactgaagacgagactgctcaaattccagctgaagcagttatcggttactctgaccttgagggtgatttcgacgtcgctgttttgcctttctctaactccactaacaacggtttgttgttcattaacaccactatcgcttccattgctgctaaggaagagggtgtctctctcgagaagagagacatcgttttgactcaatccccagctactttgtccgttactccaggtaactccgtttccttgtcctgtagagcttcccagtccatcggtaacaacttgcactggtatcagcagaagtctcacgagtccccaagactgttgatcaagtacgcttcccaatccatctccggtatcccatctagattctctggttctggttccggtactgacttcactttgtccatcaactccgttgagactgaggacttcggtatgtacttctgtcagcaatccaactcctggccatacacttttggtggtggtactaagttggagatcaagagaactgttgctgctccatccgttttcatcttcccaccatctgacgagcagttgaagtctggtactgcttccgttgtttgtttgttgaacaacttctacccaagagaagctaaggttcagtggaaggttgacaacgccttgcaatccggtaactcccaagagtccgttactgaacaagactccaaggactctacttactccttgtcctccactttgactttgtccaaggctgactacgagaagcacaaggtttacgcttgtgaggttactcaccagggtttgtcctccccagttactaagtccttcaacagaggtgagtgttaatag

SEQ ID NO: 33 - DNA, 33 bp, artificial
  Synthetic Construct
actacctgcaggcgaaacgatgagattcccatc

SEQ ID NO: 34 - DNA, 44 bp, artificial
  Synthetic Construct
tcatggccgaggcggccctattacttgtcacaggactttggctc

SEQ ID NO: 35 - DNA, 39 bp, artificial
  Synthetic Construct
ctatggccgaggcggccctattaacactcacctctgttg

SEQ ID NO: 36 - DNA, 39 bp, artificial
  Synthetic Construct
tatcggccgaggcggccctattacttacctggggacaag

SEQ ID NO: 37 - DNA, 39 bp, artificial; identical to SEQ ID NO: 35
  Synthetic Construct

SEQ ID NO: 38 - DNA, 32 bp, artificial
  Synthetic Construct
cttgcctgcaggatgctaacggccagttggtc

SEQ ID NO: 39 - DNA, 40 bp, artificial
  Synthetic Construct
gatcggccgaggcggcctcagcagtattcccaccagaatc

SEQ ID NO: 40 - DNA, 38 bp, artificial
  Synthetic Construct
cttgcctgcaggatgtcagttcatttcgttatagcagc

SEQ ID NO: 41 - DNA, 52 bp, artificial
  Synthetic Construct
gatcggccgaggcggcctcatataaaaggtttatcataattctcatcctcag

SEQ ID NO: 42 - DNA, 43 bp, artificial
  Synthetic Construct
gaaacctgcaggatgtctgaatttgttgctaaaattaacattc

SEQ ID NO: 43 - DNA, 36 bp, artificial
  Synthetic Construct
gatcggccgaggcggccttaggcggttggaacgttc

SEQ ID NO: 44 - DNA, 39 bp, artificial
  Synthetic Construct
gaaacctgcaggatgtctcatctattactgcgtgacagc

SEQ ID NO: 45 - DNA, 37 bp, artificial
  Synthetic Construct
gatcggccgaggcggcctcatggcccggcatatctag

SEQ ID NO: 46 - DNA, 43 bp, artificial
  Synthetic Construct
gacacctgcaggatgtctgaatcctccagtatctctctagttg

SEQ ID NO: 47 - DNA, 42 bp, artificial
  Synthetic Construct
gatcggccgaggcggccctagatacatcccaaaagtgcaccg

SEQ ID NO: 48 - DNA, 34 bp, artificial
  Synthetic Construct
gatacctgcaggatgatcctgggttcagtttggg

SEQ ID NO: 49 - DNA, 43 bp, artificial
  Synthetic Construct
gatcggccgaggcggccctaaaagtttgctgcagcatttgaag

SEQ ID NO: 50 - DNA, 37 bp, artificial
  Synthetic Construct
cttgcctgcaggatgggttgctttagattttgtctgg

SEQ ID NO: 51 - DNA, 42 bp, artificial
  Synthetic Construct
gatcggccgaggcggccctatttgtatacgtgctgtggagcc

SEQ ID NO: 52 - DNA, 42 bp, artificial
  Synthetic Construct
cttgcctgcaggatgttaaacaagctgttcattgcaatactc

SEQ ID NO: 53 - DNA, 41 bp, artificial
  Synthetic Construct
gatcggccgaggcggccttagctggcaagggtaattgtctc

SEQ ID NO: 54 - DNA, 33 bp, artificial
  Synthetic Construct
gacacctgcaggatggctcctcaaacaccaagg

SEQ ID NO: 55 - DNA, 44 bp, artificial
  Synthetic Construct
gatcggccgaggcggcctcaaaaaaacaatctcaaaatctccag

SEQ ID NO: 56 - DNA, 33 bp, artificial
  Synthetic Construct
gtaccctgcaggatgaccaaggaaaatgaagcc

SEQ ID NO: 57 - DNA, 41 bp, artificial
  Synthetic Construct
gatcggccgaggcggccttattttttctccaattcagccag

SEQ ID NO: 58 - DNA, 40 bp, artificial
  Synthetic Construct
gaaacctgcaggatgctgttgtcacataccatgatacttc

SEQ ID NO: 59 - DNA, 43 bp, artificial
  Synthetic Construct
gatcggccgaggcggccttaagattgcttctttttgagattgg

SEQ ID NO: 60 - DNA, 38 bp, artificial
  Synthetic Construct
gaaacctgcaggatgacggactatgtcacttctaagcg

SEQ ID NO: 61 - DNA, 37 bp, artificial
  Synthetic Construct
gatcggccgaggcggcctcataatctccctccagggg

SEQ ID NO: 62 - DNA, 33 bp, artificial
  Synthetic Construct
gaaacctgcaggatgtcgtctgatgctgtggag

SEQ ID NO: 63 - DNA, 46 bp, artificial
  Synthetic Construct
gatcggccgaggcggcctcaaataatgctacatttgcgtttctttc

SEQ ID NO: 64 - DNA, 39 bp, artificial
  Synthetic Construct
cttgcctgcaggatgtcttatacgtcggacaacaaagag

SEQ ID NO: 65 - DNA, 42 bp, artificial
  Synthetic Construct
gatcggccgaggcggccttacgtgtatccgcttcctctgtac

SEQ ID NO: 66 - DNA, 44 bp, artificial
  Synthetic Construct
gatacctgcaggatgaacttgtacctaattacattactattcgc

SEQ ID NO: 67 - DNA, 44 bp, artificial
  Synthetic Construct
gatcggccgaggcggccttagaacccacattgatttggatactg

SEQ ID NO: 68 - DNA, 37 bp, artificial
  Synthetic Construct
gaaacctgcaggatgtcgttatcaacctttctaggcg

SEQ ID NO: 69 - DNA, 47 bp, artificial
  Synthetic Construct
gatcggccgaggcggcctcagactctactcatcattttgtcttcctc

SEQ ID NO: 70 - DNA, 44 bp, artificial
  Synthetic Construct
gaaacctgcaggatgatgtacaggaacttaataattgctactgc

SEQ ID NO: 71 - DNA, 48 bp, artificial
  Synthetic Construct
gatcggccgaggcggccctaacactctatgaggtctacaatgtccaac

SEQ ID NO: 72 - DNA, 37 bp, artificial
  Synthetic Construct
catgcctgcaggatgtctacagcaattccaggaggac

SEQ ID NO: 73 - DNA, 46 bp, artificial
  Synthetic Construct
gatcggccgaggcggccttagttgatcaactttcctgtcagcttag

SEQ ID NO: 74 - DNA, 39 bp, artificial
  Synthetic Construct
gacacctgcaggatgagtggtgaccataagagctttacg

SEQ ID NO: 75 - DNA, 44 bp, artificial
  Synthetic Construct
gatcggccgaggcggccttactgtgtaccataccgatccaatcc

SEQ ID NO: 76 - DNA, 41 bp, artificial
  Synthetic Construct
cttgcctgcaggatgactaactggaaagcgatattgactcc

SEQ ID NO: 77 - DNA, 49 bp, artificial
  Synthetic Construct
gatcggccgaggcggccttagttctcttcttcaccttgaaattttaggc

SEQ ID NO: 78 - DNA, 37 bp, artificial
  Synthetic Construct
gcaacctgcaggatgtcttatcgccctcagtttcaac

SEQ ID NO: 79 - DNA, 51 bp, artificial
  Synthetic Construct
gatcggccgaggcggcctcaatagatctttttcttttcatcaaaactcaac

SEQ ID NO: 80 - DNA, 36 bp, artificial
  Synthetic Construct
gatacctgcaggatggtggtgcacaaccctaataac

SEQ ID NO: 81 - DNA, 49 bp, artificial
  Synthetic Construct
gatcggccgaggcggccctaggtactatgctgaacatcctgagtatgag

SEQ ID NO: 82 - DNA, 41 bp, artificial
  Synthetic Construct
gaaacctgcaggatgagattttctaacgtcgttttaactgc

SEQ ID NO: 83 - DNA, 42 bp, artificial
  Synthetic Construct
gatcggccgaggcggccttacaaggcaaagactccgaaagtg

SEQ ID NO: 84 - DNA, 38 bp, artificial
  Synthetic Construct
gacacctgcaggatgactgtgcctgatctgaaagaaac

SEQ ID NO: 85 - DNA, 33 bp, artificial
  Synthetic Construct
gatcggccgaggcggcctcaggccagcgcaacg

SEQ ID NO: 86 - DNA, 46 bp, artificial
  Synthetic Construct
cttgcctgcaggatgaagatatggctggtacttcttttagtttttg

SEQ ID NO: 87 - DNA, 43 bp, artificial
  Synthetic Construct
gatcggccgaggcggcctcacaattcgtctctaatttgttgcg

SEQ ID NO: 88 - DNA, 31 bp, artificial
  Synthetic Construct
cttgcctgcaggatggagcaggttccagtcg

SEQ ID NO: 89 - DNA, 47 bp, artificial
  Synthetic Construct
gatcggccgaggcggccttattcatcataaacttcttctatggtggc

SEQ ID NO: 90 - DNA, 38 bp, artificial
  Synthetic Construct
cttgcctgcaggatggatcctttttcaattcttctcac

SEQ ID NO: 91 - DNA, 47 bp, artificial
  Synthetic Construct
gatcggccgaggcggccctactttggagacagatcttccaccttaac

SEQ ID NO: 92 - DNA, 37 bp, artificial
  Synthetic Construct
gaaacctgcaggatgaccagtcaaggatttttggatc

SEQ ID NO: 93 - DNA, 49 bp, artificial
  Synthetic Construct
gatcggccgaggcggccctatatgctatcaaccatctccatcaaataac

SEQ ID NO: 94 - DNA, 36 bp, artificial
  Synthetic Construct
gacacctgcaggatgactccccgttctcatattttc

SEQ ID NO: 95 - DNA, 50 bp, artificial
  Synthetic Construct
gatcggccgaggcggccctactcaaagaacttagacaaagcagctttctc

SEQ ID NO: 96 - DNA, 29 bp, artificial
  Synthetic Construct
gatccctgcaggatggcagaagaagaacc

SEQ ID NO: 97 - DNA, 54 bp, artificial
  Synthetic Construct
gatcggccgaggcggccctaattagtaatacttgcttctatttcctggtacaac

SEQ ID NO: 98 - DNA, 40 bp, artificial
  Synthetic Construct
gaaccctgcaggatgattttgagcaagctgtcgtttagac

SEQ ID NO: 99 - DNA, 51 bp, artificial
  Synthetic Construct
gatcggccgaggcggccttatttattaacaatgacatcatcttcaaactcg

SEQ ID NO: 100 - DNA, 30 bp, artificial
  Synthetic Construct
cttgcctgcaggatgggtgccattggaatg

SEQ ID NO: 101 - DNA, 44 bp, artificial
  Synthetic Construct
gatcggccgaggcggccctattgcagaacattcgatatccaatc

SEQ ID NO: 102 - DNA, 36 bp, artificial
  Synthetic Construct
gatacctgcaggatgctaccattttcgtacgacgtg

SEQ ID NO: 103 - DNA, 45 bp, artificial
  Synthetic Construct
gatcggccgaggcggccctataactctccattctcctcgtcgatc

SEQ ID NO: 104 - DNA, 47 bp, artificial
  Synthetic Construct
gatccctgcaggatgaaaatattaagtgcattgcttcttctttttac

SEQ ID NO: 105 - DNA, 44 bp, artificial
  Synthetic Construct
gatcggccgaggcggccttatagctcttggtgtaataactgggg

SEQ ID NO: 106 - DNA, 42 bp, artificial
  Synthetic Construct
cttgcctgcaggatgtctaaaccctacaagctgataggtgag

SEQ ID NO: 107 - DNA, 45 bp, artificial
  Synthetic Construct
gatcggccgaggcggccttaatcttctccagcaggtatctcatcc

SEQ ID NO: 108 - DNA, 45 bp, artificial
  Synthetic Construct
cttgcctgcaggatgaatcaattttctctagcttcacaagtaaac

SEQ ID NO: 109 - DNA, 41 bp, artificial
  Synthetic Construct
gatcggccgaggcggccctactcggttaatggtccgagtgc

SEQ ID NO: 110 - DNA, 42 bp, artificial
  Synthetic Construct
gacacctgcaggatgagttataggaaagacaacaaacaaaag

SEQ ID NO: 111 - DNA, 39 bp, artificial
  Synthetic Construct
gatcggccgaggcggccttagaaggcagcttcatcatcg

SEQ ID NO: 112 - DNA, 40 bp, artificial
  Synthetic Construct
cttgcctgcaggatgagcagcttcagagttctagacttgg

SEQ ID NO: 113 - DNA, 35 bp, artificial
  Synthetic Construct
gatcggccgaggcggccttacagatcaacgaatcc

SEQ ID NO: 114 - DNA, 44 bp, artificial
  Synthetic Construct
gatacctgcaggatgaacatctttagaatcctaggtaagtttcc

SEQ ID NO: 115 - DNA, 39 bp, artificial
  Synthetic Construct
gatcggccgaggcggcctcattctggcagcttgaatttc

SEQ ID NO: 116 - DNA, 45 bp, artificial
  Synthetic Construct
cttgcctgcaggatgtccacaactactaagaaaaacaagaacagg

SEQ ID NO: 117 - DNA, 39 bp, artificial
  Synthetic Construct
gatcggccgaggcggccttaccatgcaccctttcctctc

SEQ ID NO: 118 - DNA, 40 bp, artificial
  Synthetic Construct
cttgcctgcaggatgtcagaggagtaagaaccacaaacag

SEQ ID NO: 119 - DNA, 45 bp, artificial
  Synthetic Construct
gatcggccgaggcggcctcaatttattctaggttttttggttcgg

SEQ ID NO: 120 - DNA, 31 bp, artificial
  Synthetic Construct
gtaccctgcaggatgatggcaagtccaaccg

SEQ ID NO: 121 - DNA, 34 bp, artificial
  Synthetic Construct
gatcggccgaggcggcccgcaacaacgctggttg

SEQ ID NO: 122 - DNA, 42 bp, artificial
  Synthetic Construct
cttgcctgcaggatgagtaaccagtataatccgtatgagcag

SEQ ID NO: 123 - DNA, 40 bp, artificial
  Synthetic Construct
gatcggccgaggcggccctatcttccccagtttccgacac

SEQ ID NO: 124 - DNA, 43 bp, artificial
  Synthetic Construct
gttacctgcaggatgtctacagagaacaaagcagagacaaaac

SEQ ID NO: 125 - DNA, 41 bp, artificial
  Synthetic Construct
gatcggccgaggcggccctatttctttgcttcagcgtttgc

SEQ ID NO: 126 - DNA, 44 bp, artificial
  Synthetic Construct
cttgcctgcaggatgttaaacttaatatccacaataagtgggtg

SEQ ID NO: 127 - DNA, 41 bp, artificial
  Synthetic Construct
gatcggccgaggcggccttaagcaggagcagataaccaagc

SEQ ID NO: 128 - DNA, 42 bp, artificial
  Synthetic Construct
cttgcctgcaggatgggtagaaggaaaatagagataaatccg

SEQ ID NO: 129 - DNA, 43 bp, artificial
  Synthetic Construct
gatcggccgaggcggcctcagctcttcttagtcacactgcttg

SEQ ID NO: 130 - DNA, 40 bp, artificial
  Synthetic Construct
cttgcctgcaggatgtcacttcaactgtccattatcttcg

SEQ ID NO: 131 - DNA, 44 bp, artificial
  Synthetic Construct
gatcggccgaggcggccctactcgtccttcttgttgctcttctc

SEQ ID NO: 132 - DNA, 22 bp, artificial
  Synthetic Construct
cgaacatccatcaccaaaacac

SEQ ID NO: 133 - DNA, 37 bp, artificial
  Synthetic Construct
gttgtcgacctgcagcgtacggtgttgccgcgaaatg

SEQ ID NO: 134 - DNA, 37 bp, artificial
  Synthetic Construct
catttcgcggcaacaccgtacgctgcaggtcgacaac

SEQ ID NO: 135 - DNA, 24 bp, artificial
  Synthetic Construct
cggtgagaatggcaaaagcttatg

SEQ ID NO: 136 - DNA, 21 bp, artificial
  Synthetic Construct
aagcccgatgcgccagagttg

SEQ ID NO: 137 - DNA, 41 bp, artificial
  Synthetic Construct
cgtctcttgggcaaattgatcagtggatctgatatcaccta

SEQ ID NO: 138 - DNA, 41 bp, artificial
  Synthetic Construct
taggtgatatcagatccactgatcaatttgcccaagagacg

SEQ ID NO: 139 - DNA, 20 bp, artificial
  Synthetic Construct
gactgttgcgattgctggtg

SEQ ID NO: 140 - DNA, 21 bp, artificial
  Synthetic Construct
atccaggacacgctcatcaag

SEQ ID NO: 141 - DNA, 22 bp, artificial
  Synthetic Construct
gtgtgtgctctggaattggatc

SEQ ID NO: 142 - DNA, 23 bp, artificial
  Synthetic Construct
agaggaggttgaatgcgaagaag

SEQ ID NO: 143 - DNA, 49 bp, artificial
  Synthetic Construct
gttgtcgacctgcagcgtacttctggtgagcttatatggcagtagttac

SEQ ID NO: 144 - DNA, 49 bp, artificial
  Synthetic Construct
gtaactactgccatataagctcaccagaagtacgctgcaggtcgacaac

SEQ ID NO: 145 - DNA, 24 bp, artificial
  Synthetic Construct
cggtgagaatggcaaaagcttatg

SEQ ID NO: 146 - DNA, 21 bp, artificial
  Synthetic Construct
aagcccgatgcgccagagttg

SEQ ID NO: 147 - DNA, 39 bp, artificial
  Synthetic Construct
ctcgggatcaccaagcacaagtggatctgatatcaccta

SEQ ID NO: 148 - DNA, 39 bp, artificial
  Synthetic Construct
taggtgatatcagatccacttgtgcttggtgatcccgag

SEQ ID NO: 149 - DNA, 23 bp, artificial
  Synthetic Construct
tcaaagtatgctgggaagaatgg

SEQ ID NO: 150 - DNA, 18 bp, artificial
  Synthetic Construct
tggattgtctcggaggcg

SEQ ID NO: 151 - DNA, 26 bp, artificial
  Synthetic Construct
tactatgactatgggagacctgggtg

SEQ ID NO: 152 - DNA, 19 bp, artificial
  Synthetic Construct
tgaagcatcccacccactg

SEQ ID NO: 153 - DNA, 44 bp, artificial
  Synthetic Construct
gttgtcgacctgcagcgtacccttcgcagactgtaattattggc

SEQ ID NO: 154 - DNA, 44 bp, artificial
  Synthetic Construct
gccaataattacagtctgcgaagggtacgctgcaggtcgacaac

SEQ ID NO: 155 - DNA, 24 bp, artificial
  Synthetic Construct
cggtgagaatggcaaaagcttatg

SEQ ID NO: 156 - DNA, 21 bp, artificial
  Synthetic Construct
aagcccgatgcgccagagttg

SEQ ID NO: 157 - DNA, 44 bp, artificial
  Synthetic Construct
gttgactttgacggttgcagatacagtggatctgatatcaccta

SEQ ID NO: 158 - DNA, 44 bp, artificial
  Synthetic Construct
taggtgatatcagatccactgtatctgcaaccgtcaaagtcaac

SEQ ID NO: 159 - DNA, 27 bp, artificial
  Synthetic Construct
ttctctccttgattatcggtctctttc

SEQ ID NO: 160 - DNA, 21 bp, artificial
  Synthetic Construct
tggcagatgacttcacaaacg

SEQ ID NO: 161 - DNA, 25 bp, artificial
  Synthetic Construct
gtggcatctttcataacgacatctc

SEQ ID NO: 162 - protein, 478 aa, Pichia pastoris
MSSFRVLDLVKPFTPFLPEVISPERKVPFQQKLMWTGVTLLIFLVMSEIPLYGITSSDSSDPLFWLRMMLASNRGTLMELGISPIVTSGMVFQLLQGIQILDVNMENKADRELFQTAQKVFAILLSIGQATVYVLTGMYGPPGELGVGVCLLLVLQLVFAGIVVILLDELLQKGYGLGSGISLFMATNICEQIFWKTFAPTTVNRGRGKEFEGAFISFFHLILTKKDKKRALLESFYRDNAPNMFQVIATLVVFFTVVYLQGFRLEIPVKSTRQRGPYGTYPIRLFYTSNMPIMLQSALTSNIFIISQMLYSHFPDNAFVKLIGTWEAQPGSAQLFAASGLAYYMQPPMSLSQALLDPIKTVVYVVFVLTTCAIFSKTWIEISGSSPRDVAKQFKDQGLVIAGHRDATVYKELKKIIPTAAAFGGATIGALSVVSDLLGTLGSGTSILLAVTTIYGYYELAVKEGGFSKGGPSGFVDL

SEQ ID NO: 163 - DNA, 1437 bp, Pichia pastoris
atgagcagcttcagagttctagacttggtaaagccctttaccccatttctgcctgaggttatctctccagagagaaaggtcccctttcaacagaagttgatgtggactggagtcactcttctgatcttcttggtcatgagtgaaattcccctgtatggtatcacttcaagtgactcctctgaccctttgttttggctgcgtatgatgttggcctctaacagaggaacgctgatggagttaggtatctctcctattgtcacttctggaatggtgttccaactgttgcagggaatccaaatcttggacgtgaacatggaaaacaaagcagacagagagttgttccaaactgctcaaaaagtgttcgccattttgctgagtatcggacaagctactgtttatgttttaactggaatgtatggcccccctggtgaactaggagttggtgtctgtcttttgttggttcttcaattggtgtttgcaggtattgtggtcattttgttggatgaactcttacaaaaaggttacggtttaggaagtggaatttctcttttcatggccaccaacatttgtgagcagattttttggaagacttttgctcctaccaccgttaaccgtggaagaggtaaggaatttgaaggagctttcatttctttctttcacctgatcttgaccaagaaggacaagaagagagctctgttggaatcattttacagagacaacgctccaaacatgttccaagttattgctactcttgtcgtctttttcaccgttgtctatcttcagggcttccgtttggagattccagttaagtctacccgtcaaagaggtccttacggaacttacccaatcagattgttctacacatccaacatgccaatcatgttacaatccgctttgacctcaaacattttcattatttcccagatgttgtattcacacttccctgacaatgcctttgttaagctcattggaacttgggaagctcaacctggttcagcacaactgtttgctgcctcgggattagcctactacatgcagcctccaatgtccctgagtcaagctttattagaccctatcaagactgtcgtctacgttgtgtttgttttgaccacttgtgccatcttctccaagacatggattgagatttcgggatcttccccaagagacgttgctaagcaattcaaagaccaaggattggttattgctggacacagagatgctactgtttacaaggagttgaagaagattataccaacagccgctgcatttggaggtgccacaattggtgcactttccgttgtttccgaccttttgggtactttaggttcgggaacctccatccttttggctgttacaaccatctatggttactacgagttggctgttaaggaaggtggtttttcaaagggtggaccctctggattcgttgatctgtaa